European Patent Application EP 4 585 228 A2, published July 16, 2025. Title: DOSING REGIMENS AND RELATED COMPOSITIONS AND METHODS. Applicant: APELLIS PHARMACEUTICALS, INC. Application EP. The sequence listing filed with the application follows.

SEQUENCE LISTING (74 sequences)

SEQ ID NO: 1 - protein, 13 aa, synthetic construct
  REGION 1..13: note = Description of Artificial Sequence: Synthetic peptide
  DISULFID 2..12: note = Disulfide bond
ICVVQDWGHHRCT

SEQ ID NO: 2-5 - skipped (4 entries)

SEQ ID NO: 6 - protein, 16 aa, synthetic construct
  VARIANT 1..2: note = Ile, Val, Leu, B1-Ile, B1-Val, B1-Leu or a dipeptide comprising Gly-Ile or B1-Gly-Ile, wherein B1 represents a first blocking moiety. This region may encompass 1 to 2 residues, wherein some positions may be absent.
  DISULFID 3..13: note = Disulfide bond
  VARIANT 5: note = Independently selected from Trp or analogs of Trp
  VARIANT 8: note = Independently selected from Trp or analogs of Trp
  VARIANT 10: note = His, Ala or an analog of Ala, Phe, Trp or an analog of Trp
  VARIANT 14..16: note = L-Thr, D-Thr, Ile, Val, Gly, a dipeptide selected from Thr-Ala or Thr-Asn, or a tripeptide comprising Thr-Ala-Asn, wherein a c-term -OH of any of the L-Thr, D-Thr, Ile, Val, Gly, Ala or Asn is optionally replaced by a second blocking moiety. This region may encompass 1 to 3 residues, wherein some positions may be absent.
  REGION 1..16: note = See specification as filed for detailed description of substitutions and preferred embodiments
XXCVXQDXGXHRCXXX

SEQ ID NO: 7 - protein, 16 aa, synthetic construct
  VARIANT 1..2: note = Ile, Val, Leu, Ac-Ile, Ac-Val, Ac-Leu, a dipeptide comprising Gly-Ile or Ac-Gly-Ile. This region may encompass 1 to 2 residues, wherein some positions may be absent.
  DISULFID 3..13: note = Disulfide bond
  VARIANT 5: note = Independently selected from Trp or analogs of Trp
  VARIANT 8: note = Independently selected from Trp or analogs of Trp
  VARIANT 10: note = His, Ala or an analog of Ala, Phe, Trp or an analog of Trp
  VARIANT 14..16: note = L-Thr, D-Thr, Ile, Val, Gly, a dipeptide selected from Thr-Ala or Thr-Asn, or a tripeptide comprising Thr-Ala-Asn, wherein a c-term -OH of any of L-Thr, D-Thr, Ile, Val, Gly, Ala, or Asn is optionally replaced by -NH2. This region may encompass 1 to 3 residues, wherein some positions may be absent.
  REGION 1..16: note = See specification as filed for detailed description of substitutions and preferred embodiments
XXCVXQDXGXHRCXXX

SEQ ID NO: 8 - protein, 13 aa, synthetic construct
  REGION 1..13: note = Description of Artificial Sequence: Synthetic peptide
  SITE 1: note = N-terminus -H
  SITE 13: note = Amidated C-terminus
ICVVQDWGHHRCT

SEQ ID NO: 9 - protein, 13 aa, synthetic construct
  REGION 1..13: note = Description of Artificial Sequence: Synthetic peptide
  SITE 1: note = Acetylated N-terminus
  SITE 13: note = Amidated C-terminus
ICVVQDWGHHRCT

SEQ ID NO: 10 - protein, 13 aa, synthetic construct
  REGION 1..13: note = Description of Artificial Sequence: Synthetic peptide
  SITE 1: note = Acetylated N-terminus
  SITE 13: note = Amidated C-terminus
ICVYQDWGAHRCT

SEQ ID NO: 11 - protein, 13 aa, synthetic construct
  REGION 1..13: note = Description of Artificial Sequence: Synthetic peptide
  SITE 1: note = Acetylated N-terminus
  SITE 13: note = Carboxylated C-terminus
ICVWQDWGAHRCT

SEQ ID NO: 12 - protein, 13 aa, synthetic construct
  REGION 1..13: note = Description of Artificial Sequence: Synthetic peptide
  SITE 1: note = Acetylated N-terminus
  SITE 13: note = Amidated C-terminus
ICVWQDWGAHRCT

SEQ ID NO: 13 - protein, 13 aa, synthetic construct
  REGION 1..13: note = Description of Artificial Sequence: Synthetic peptide
  SITE 1: note = Acetylated N-terminus
  SITE 13: note = D-Threonine
  SITE 13: note = Carboxylated C-terminus
ICVWQDWGAHRCT

SEQ ID NO: 14 - protein, 13 aa, synthetic construct
  REGION 1..13: note = Description of Artificial Sequence: Synthetic peptide
  SITE 1: note = Acetylated N-terminus
  SITE 4: note = 2-naphthylalanine
  SITE 13: note = Amidated C-terminus
ICVAQDWGAHRCT

SEQ ID NO: 15 - protein, 13 aa, synthetic construct
  REGION 1..13: note = Description of Artificial Sequence: Synthetic peptide
  SITE 1: note = Acetylated N-terminus
  SITE 4: note = 2-naphthylalanine
  SITE 13: note = Carboxylated C-terminus
ICVAQDWGAHRCT

SEQ ID NO: 16 - protein, 13 aa, synthetic construct
  REGION 1..13: note = Description of Artificial Sequence: Synthetic peptide
  SITE 1: note = Acetylated N-terminus
  SITE 4: note = 1-naphthylalanine
  SITE 13: note = Carboxylated C-terminus
ICVAQDWGAHRCT

SEQ ID NO: 17 - protein, 13 aa, synthetic construct
  REGION 1..13: note = Description of Artificial Sequence: Synthetic peptide
  SITE 1: note = Acetylated N-terminus
  SITE 4: note = 2- indanylglycine carboxylic acid
  SITE 13: note = Amidated C-terminus
ICVGQDWGAHRCT

SEQ ID NO: 18 - protein, 13 aa, synthetic construct
  REGION 1..13: note = Description of Artificial Sequence: Synthetic peptide
  SITE 1: note = Acetylated N-terminus
  SITE 4: note = 2- indanylglycine carboxylic acid
  SITE 13: note = Carboxylated C-terminus
ICVGQDWGAHRCT

SEQ ID NO: 19 - protein, 13 aa, synthetic construct
  REGION 1..13: note = Description of Artificial Sequence: Synthetic peptide
  SITE 1: note = Acetylated N-terminus
  SITE 4: note = Dihydrotrpytophan
  SITE 1..13: note = Carboxylated C-terminus
ICVWQDWGAHRCT

SEQ ID NO: 20 - protein, 13 aa, synthetic construct
  REGION 1..13: note = Description of Artificial Sequence: Synthetic peptide
  SITE 1: note = Acetylated N-terminus
  SITE 4: note = 4-benzoyl-L-phenylalanine
  SITE 13: note = Carboxylated C-terminus
ICVFQDWGAHRCT

SEQ ID NO: 21 - protein, 13 aa, synthetic construct
  REGION 1..13: note = Description of Artificial Sequence: Synthetic peptide
  SITE 1: note = Acetylated N-terminus
  SITE 4: note = 4-benzoyl-L-phenylalanine
  SITE 13: note = Amidated C-terminus
ICVFQDWGAHRCT

SEQ ID NO: 22 - protein, 13 aa, synthetic construct
  REGION 1..13: note = Description of Artificial Sequence: Synthetic peptide
  SITE 1: note = Acetylated N-terminus
  SITE 4: note = Bta
  SITE 13: note = Carboxylated C-terminus
ICVXQDWGAHRCT

SEQ ID NO: 23 - protein, 13 aa, synthetic construct
  REGION 1..13: note = Description of Artificial Sequence: Synthetic peptide
  SITE 1: note = Acetylated N-terminus
  SITE 4: note = Bta
  SITE 13: note = Amidated C-terminus
ICVXQDWGAHRCT

SEQ ID NO: 24 - protein, 13 aa, synthetic construct
  REGION 1..13: note = Description of Artificial Sequence: Synthetic peptide
  SITE 1: note = Acetylated N-terminus
  SITE 9: note = 2-alpha-aminobutyric acid
  SITE 13: note = Amidated C-terminus
ICVWQDWGXHRCT

SEQ ID NO: 25 - protein, 16 aa, synthetic construct
  REGION 1..16: note = Description of Artificial Sequence: Synthetic peptide
  SITE 1: note = N-terminus -H
  SITE 16: note = Carboxylated C-terminus
GICVWQDWGAHRCTAN

SEQ ID NO: 26 - protein, 13 aa, synthetic construct
  REGION 1..13: note = Description of Artificial Sequence: Synthetic peptide
  SITE 1: note = Acetylated N-terminus
  SITE 4: note = 5-fluorotryptophan
  SITE 13: note = Amidated C-terminus
ICVWQDWGAHRCT

SEQ ID NO: 27 - protein, 13 aa, synthetic construct
  REGION 1..13: note = Description of Artificial Sequence: Synthetic peptide
  SITE 1: note = Acetylated N-terminus
  SITE 4: note = 5-methyltryptophan
  SITE 13: note = Amidated C-terminus
ICVWQDWGAHRCT

SEQ ID NO: 28 - protein, 13 aa, synthetic construct
  REGION 1..13: note = Description of Artificial Sequence: Synthetic peptide
  SITE 1: note = Acetylated N-terminus
  SITE 4: note = 1-methyltryptophan
  SITE 13: note = Amidated C-terminus
ICVWQDWGAHRCT

SEQ ID NO: 29 - protein, 13 aa, synthetic construct
  REGION 1..13: note = Description of Artificial Sequence: Synthetic peptide
  SITE 1: note = Acetylated N-terminus
  SITE 7: note = 5-fluorotryptophan
  SITE 13: note = Amidated C-terminus
ICVWQDWGAHRCT

SEQ ID NO: 30 - protein, 13 aa, synthetic construct
  REGION 1..13: note = Description of Artificial Sequence: Synthetic peptide
  SITE 1: note = Acetylated N-terminus
  SITE 4: note = 5-fluorotryptophan
  SITE 7: note = 5-fluorotryptophan
  SITE 13: note = Amidated C-terminus
ICVWQDWGAHRCT

SEQ ID NO: 31 - protein, 13 aa, synthetic construct
  REGION 1..13: note = Description of Artificial Sequence: Synthetic peptide
  SITE 1: note = Acetylated N-terminus
  SITE 4: note = 5-methyltryptophan
  SITE 7: note = 5-fluorotryptophan
  SITE 13: note = Amidated C-terminus
ICVWQDWGAHRCT

SEQ ID NO: 32 - protein, 13 aa, synthetic construct
  REGION 1..13: note = Description of Artificial Sequence: Synthetic peptide
  SITE 1: note = Acetylated N-terminus
  SITE 4: note = 1-methyltryptophan
  SITE 7: note = 5-fluorotryptophan
  SITE 13: note = Amidated C-terminus
ICVWQDWGAHRCT

SEQ ID NO: 33 - protein, 15 aa, synthetic construct
  REGION 1..15: note = Description of Artificial Sequence: Synthetic peptide
  SITE 1: note = N-terminus -H
  SITE 5: note = 6-fluorotryptophan
  SITE 8: note = 6-fluorotryptophan
  SITE 15: note = Carboxylated C-terminus
GICVWQDWGAHRCTN

SEQ ID NO: 34 - protein, 13 aa, synthetic construct
  REGION 1..13: note = Description of Artificial Sequence: Synthetic peptide
  SITE 1: note = Acetylated N-terminus
  SITE 4: note = 1-formyl-tryptophan
  SITE 13: note = Amidated C-terminus
ICVWQDWGAHRCT

SEQ ID NO: 35 - protein, 13 aa, synthetic construct
  REGION 1..13: note = Description of Artificial Sequence: Synthetic peptide
  SITE 1: note = Acetylated N-terminus
  SITE 4: note = 1-methoxy-tryptophan
  SITE 13: note = Amidated C-terminus
ICVWQDWGAHRCT

SEQ ID NO: 36 - protein, 15 aa, synthetic construct
  REGION 1..15: note = Description of Artificial Sequence: Synthetic peptide
  SITE 1: note = N-terminus -H
  SITE 5: note = 5-fluorotryptophan
  SITE 8: note = 5-fluorotryptophan
  SITE 15: note = Carboxylated C-terminus
GICVWQDWGAHRCTN

SEQ ID NO: 37 - protein, 13 aa, synthetic construct
  REGION 1..13: note = Description of Artificial Sequence: Synthetic peptide
  DISULFID 2..12: note = Disulfide bond
  SITE 4: note = 1-methyltryptophan
ICVWQDWGAHRCT

SEQ ID NO: 38 - protein, 13 aa, synthetic construct
  REGION 1..13: note = Description of Artificial Sequence: Synthetic peptide
  SITE 1: note = N-term Maleimide-(CH2)5-C(=O)
  DISULFID 2..12: note = Disulfide bond
  SITE 4: note = 1-methyltryptophan
  SITE 13: note = C-terminal amination -NH2
ICVWQDWGAHRCT

SEQ ID NO: 39 - protein, 13 aa, synthetic construct
  REGION 1..13: note = Description of Artificial Sequence: Synthetic peptide
  SITE 1: note = Acetylated N-terminus
  DISULFID 2..12: note = Disulfide bond
  SITE 4: note = 1-methyltryptophan
  SITE 13: note = C-terminus (C=O)-(CH2)5-maleimide
ICVWQDWGAHRCT

SEQ ID NO: 40 - protein, 13 aa, synthetic construct
  REGION 1..13: note = Description of Artificial Sequence: Synthetic peptide
  SITE 1: note = N-term Maleimide-(CH2)2-C(=O)-NH-CH2CH2OCH2CH2O CH2CH2C(=O)
  DISULFID 2..12: note = Disulfide bond
  SITE 4: note = 1-methyltryptophan
  SITE 13: note = C-terminal amination -NH2
ICVWQDWGAHRCT

SEQ ID NO: 41 - protein, 13 aa, synthetic construct
  REGION 1..13: note = Description of Artificial Sequence: Synthetic peptide
  SITE 1: note = N-term Maleimide-(CH2)2-C(=O)-NH-CH2CH2OCH2CH2C(=O)
  DISULFID 2..12: note = Disulfide bond
  SITE 4: note = 1-methyltryptophan
  SITE 13: note = C-terminal amination -NH2
ICVWQDWGAHRCT

SEQ ID NO: 42 - protein, 13 aa, synthetic construct
  REGION 1..13: note = Description of Artificial Sequence: Synthetic peptide
  SITE 1: note = N-term Maleimide-(CH2)3-C(=O)-NH-CH2CH2OCH2CH2 OCH2C(=O)
  DISULFID 2..12: note = Disulfide bond
  SITE 4: note = 1-methyltryptophan
  SITE 13: note = C-terminal amination -NH2
ICVWQDWGAHRCT

SEQ ID NO: 43 - protein, 13 aa, synthetic construct
  REGION 1..13: note = Description of Artificial Sequence: Synthetic peptide
  SITE 1: note = N-term Maleimide-(CH2)5-C(=O)-NH-CH2CH2OCH2CH2 OCH2C(=O)
  DISULFID 2..12: note = Disulfide bond
  SITE 4: note = 1-methyltryptophan
  SITE 13: note = C-terminal amination -NH2
ICVWQDWGAHRCT

SEQ ID NO: 44 - protein, 13 aa, synthetic construct
  REGION 1..13: note = Description of Artificial Sequence: Synthetic peptide
  SITE 1: note = N-term Maleimide-(CH2)4-C(=O)-NH-CH2CH2OCH2CH2 OCH2CH2C(=O)
  DISULFID 2..12: note = Disulfide bond
  SITE 4: note = 1-methyltryptophan
  SITE 13: note = C-terminal amination -NH2
ICVWQDWGAHRCT

SEQ ID NO: 45 - protein, 13 aa, synthetic construct
  REGION 1..13: note = Description of Artificial Sequence: Synthetic peptide
  SITE 1: note = N-term Maleimide-(CH2)2-C(=O)-NH-CH2CH2OCH2CH2 OCH2CH2C(=O)
  DISULFID 2..12: note = Disulfide bond
  SITE 4: note = 1-methyltryptophan
  SITE 13: note = C-terminal amination -NH2
ICVWQDWGAHRCT

SEQ ID NO: 46 - protein, 13 aa, synthetic construct
  REGION 1..13: note = Description of Artificial Sequence: Synthetic peptide
  SITE 1: note = N-term Maleimide-(CH2)5-C(=O)-NH-CH2CH2OCH2CH2 OCH2C(=O)
  DISULFID 2..12: note = Disulfide bond
  SITE 4: note = 1-methyltryptophan
  SITE 13: note = C-terminal amination -NH2
ICVWQDWGAHRCT

SEQ ID NO: 47 - protein, 14 aa, synthetic construct
  REGION 1..14: note = Description of Artificial Sequence: Synthetic peptide
  SITE 1: note = Acetylated N-terminus
  DISULFID 2..12: note = Disulfide bond
  SITE 4: note = 1-methyltryptophan
  SITE 14: note = C-terminal amination -NH2
ICVWQDWGAHRCTK

SEQ ID NO: 48 - protein, 19 aa, synthetic construct
  REGION 1..19: note = Description of Artificial Sequence: Synthetic peptide
  SITE 1: note = Acetylated N-terminus
  DISULFID 2..12: note = Disulfide bond
  SITE 4: note = 1-methyltryptophan
  SITE 19: note = C-terminal amination -NH2
ICVWQDWGAHRCTGGGGGK

SEQ ID NO: 49 - protein, 13 aa, synthetic construct
  REGION 1..13: note = Description of Artificial Sequence: Synthetic peptide
  SITE 1: note = N-term NH2(CH2)5C(=O)
  SITE 4: note = 1-methyltryptophan
  SITE 13: note = C-terminal amination -NH2
ICVWQDWGAHRCT

SEQ ID NO: 50 - protein, 13 aa, synthetic construct
  REGION 1..13: note = Description of Artificial Sequence: Synthetic peptide
  SITE 1: note = N-term NH2(CH2CH2O)2CH2C(=O)
  SITE 4: note = 1-methyltryptophan
  SITE 13: note = C-terminal amination -NH2
ICVWQDWGAHRCT

SEQ ID NO: 51 - protein, 14 aa, synthetic construct
  REGION 1..14: note = Description of Artificial Sequence: Synthetic peptide
  SITE 1: note = Acetylated N-terminus
  DISULFID 2..12: note = Disulfide bond
  SITE 4: note = 1-methyltryptophan
  MOD_RES 14: note = NH-CH2CH2OCH2CH2OCH2-C(=O)-Lys
  SITE 14: note = C-terminal amination -NH2
ICVWQDWGAHRCTK

SEQ ID NO: 52 - protein, 14 aa, synthetic construct
  REGION 1..14: note = Description of Artificial Sequence: Synthetic peptide
  SITE 1: note = Acetylated N-terminus
  DISULFID 2..12: note = Disulfide bond
  SITE 4: note = 1-methyltryptophan
  MOD_RES 14: note = Lys-(C(=O)-(CH2)5-Mal)
  SITE 14: note = C-terminal amination -NH2
ICVWQDWGAHRCTK

SEQ ID NO: 53 - protein, 19 aa, synthetic construct
  REGION 1..19: note = Description of Artificial Sequence: Synthetic peptide
  SITE 1: note = Acetylated N-terminus
  DISULFID 2..12: note = Disulfide bond
  SITE 4: note = 1-methyltryptophan
  MOD_RES 19: note = Lys-(C(=O)-(CH2)5-Mal)
  SITE 19: note = C-terminal amination -NH2
ICVWQDWGAHRCTGGGGGK

SEQ ID NO: 54 - protein, 13 aa, synthetic construct
  REGION 1..13: note = Description of Artificial Sequence: Synthetic peptide
  SITE 1: note = N-term Mal-(CH2)5-(C(=O)-NH(CH2)5C(=O)
  SITE 4: note = 1-methyltryptophan
  SITE 13: note = C-terminal amination -NH2
ICVWQDWGAHRCT

SEQ ID NO: 55 - protein, 13 aa, synthetic construct
  REGION 1..13: note = Description of Artificial Sequence: Synthetic peptide
  SITE 1: note = N-term Mal-(CH2)5-(C(=O)NH(CH2CH2O)2CH2C(=O)
  SITE 4: note = 1-methyltryptophan
  SITE 13: note = C-terminal amination -NH2
ICVWQDWGAHRCT

SEQ ID NO: 56 - protein, 14 aa, synthetic construct
  REGION 1..14: note = Description of Artificial Sequence: Synthetic peptide
  SITE 1: note = Acetylated N-terminus
  DISULFID 2..12: note = Disulfide bond
  SITE 4: note = 1-methyltryptophan
  MOD_RES 14: note = NH-CH2CH2OCH2CH2OCH2-C(=O)-Lys-(C(=O)-(CH2)5-Mal)
  SITE 14: note = C-terminal amination -NH2
ICVWQDWGAHRCTK

SEQ ID NO: 57 - protein, 14 aa, synthetic construct
  REGION 1..14: note = Description of Artificial Sequence: Synthetic peptide
  SITE 1: note = Acetylated N-terminus
  DISULFID 2..12: note = Disulfide bond
  SITE 4: note = 1-methyltryptophan
  MOD_RES 14: note = Lys-C(=O)-CH2(OCH2CH2)2NH(C(=O)-(CH2)5-Mal)
  SITE 14: note = C-terminal amination -NH2
ICVWQDWGAHRCTK

SEQ ID NO: 58 - protein, 13 aa, synthetic construct
  REGION 1..13: note = Description of Artificial Sequence: Synthetic peptide
  SITE 1: note = N-term (CH2CH2O)nC(=O)
  SITE 4: note = 1-methyltryptophan
  SITE 13: note = C-terminal amination -NH2
  REGION 1..13: note = See specification as filed for detailed description of substitutions and preferred embodiments
ICVWQDWGAHRCT

SEQ ID NO: 59 - protein, 14 aa, synthetic construct
  REGION 1..14: note = Description of Artificial Sequence: Synthetic peptide
  SITE 1: note = Acetylated N-terminus
  DISULFID 2..12: note = Disulfide bond
  SITE 4: note = 1-methyltryptophan
  MOD_RES 14: note = NH-CH2CH2OCH2CH2OCH2-C(=O)-Lys-C(=O)-(CH2CH2O)n
  SITE 14: note = C-terminal amination -NH2
  REGION 1..14: note = See specification as filed for detailed description of substitutions and preferred embodiments
ICVWQDWGAHRCTK

SEQ ID NO: 60 - protein, 14 aa, synthetic construct
  REGION 1..14: note = Description of Artificial Sequence: Synthetic peptide
  SITE 1: note = Acetylated N-terminus
  DISULFID 2..12: note = Disulfide bond
  SITE 4: note = 1-methyltryptophan
  MOD_RES 14: note = Lys-C(=O)-(CH2CH2O)n
  SITE 14: note = C-terminal amination -NH2
  REGION 1..14: note = See specification as filed for detailed description of substitutions and preferred embodiments
ICVWQDWGAHRCTK

SEQ ID NO: 61 - protein, 19 aa, synthetic construct
  REGION 1..19: note = Description of Artificial Sequence: Synthetic peptide
  SITE 1: note = Acetylated N-terminus
  DISULFID 2..12: note = Disulfide bond
  SITE 4: note = 1-methyltryptophan
  MOD_RES 19: note = Lys-C(=O)-(CH2CH2O)n
  SITE 19: note = C-terminal amination -NH2
  REGION 1..19: note = See specification as filed for detailed description of substitutions and preferred embodiments
ICVWQDWGAHRCTGGGGGK

SEQ ID NO: 62 - protein, 19 aa, synthetic construct
  REGION 1..19: note = Description of Artificial Sequence: Synthetic peptide
  SITE 1: note = Acetylated N-terminus
  MOD_RES 1: note = (CH2CH2O)nC(=O)Lys
  DISULFID 8..18: note = Disulfide bond
  SITE 10: note = 1-methyltryptophan
  SITE 19: note = C-terminal amination -NH2
  REGION 1..19: note = See specification as filed for detailed description of substitutions and preferred embodiments
KGGGGGICVWQDWGAHRCT

SEQ ID NO: 63 - protein, 14 aa, synthetic construct
  REGION 1..14: note = Description of Artificial Sequence: Synthetic peptide
  SITE 1: note = Acetylated N-terminus
  MOD_RES 1: note = (CH2CH2O)nC(=O)Lys
  DISULFID 3..13: note = Disulfide bond
  SITE 5: note = 1-methyltryptophan
  SITE 14: note = C-terminal amination -NH2
  REGION 1..14: note = See specification as filed for detailed description of substitutions and preferred embodiments
KICVWQDWGAHRCT

SEQ ID NO: 64 - protein, 14 aa, synthetic construct
  REGION 1..14: note = Description of Artificial Sequence: Synthetic peptide
  SITE 1: note = Acetylated N-terminus
  DISULFID 2..12: note = Disulfide bond
  SITE 4: note = 1-methyltryptophan
  MOD_RES 14: note = NH-CH2CH2OCH2CH2OCH2-C(=O)-Lys-(C(=O)-(CH2CH2O)n-R)
  SITE 14: note = C-terminal amination -NH2
  REGION 1..14: note = See specification as filed for detailed description of substitutions and preferred embodiments
ICVWQDWGAHRCTK

SEQ ID NO: 65 - protein, 14 aa, synthetic construct
  REGION 1..14: note = Description of Artificial Sequence: Synthetic peptide
  SITE 1: note = Acetylated N-terminus
  DISULFID 2..12: note = Disulfide bond
  SITE 4: note = 1-methyltryptophan
  MOD_RES 14: note = NH-CH2CH2OCH2CH2OCH2-C(=O)-Lys-(C(=O)-(CH2)m- (CH2CH2O)n-R)
  SITE 14: note = C-terminal amination -NH2
  REGION 1..14: note = See specification as filed for detailed description of substitutions and preferred embodiments
ICVWQDWGAHRCTK

SEQ ID NO: 66 - protein, 14 aa, synthetic construct
  REGION 1..14: note = Description of Artificial Sequence: Synthetic peptide
  SITE 1: note = Acetylated N-terminus
  SITE 2..12: note = Disulfide bond
  SITE 4: note = 1-methyltryptophan
  MOD_RES 14: note = NH-CH2CH2OCH2CH2OCH2-C(=O)-Lys-(C(=O)-(CH2)m-C(=O)- (CH2CH2O)n-R)
  SITE 14: note = C-terminal amination -NH2
  REGION 1..14: note = See specification as filed for detailed description of substitutions and preferred embodiments
ICVWQDWGAHRCTK

SEQ ID NO: 67 - protein, 14 aa, synthetic construct
  REGION 1..14: note = Description of Artificial Sequence: Synthetic peptide
  SITE 1: note = Acetylated N-terminus
  DISULFID 2..12: note = Disulfide bond
  SITE 4: note = 1-methyltryptophan
  MOD_RES 14: note = NH-CH2CH2OCH2CH2OCH2-C(=O)-Lys-(C(=O)-(CH2)m-C(=O) -(CH2)j(CH2CH2O)n-R)
  SITE 14: note = C-terminal amination -NH2
ICVWQDWGAHRCTK

SEQ ID NO: 68 - protein, 14 aa, synthetic construct
  REGION 1..14: note = Description of Artificial Sequence: Synthetic peptide
  SITE 1: note = Acetylated N-terminus
  DISULFID 2..12: note = Disulfide bond
  SITE 4: note = 1-methyltryptophan
  SITE 13..14: note = Residues at these positions are linked by an AEEAc moiety
  MOD_RES 14: note = Lys-(C(=O)-(CH2)5-Mal)
  SITE 14: note = C-terminal amination -NH2
ICVWQDWGAHRCTK

SEQ ID NO: 69 - protein, 6 aa, synthetic construct
  REGION 1..6: note = Description of Artificial Sequence: Synthetic 6xHis tag
HHHHHH

SEQ ID NO: 70 - skipped

SEQ ID NO: 71 - protein, 18 aa, synthetic construct
  REGION 1..18: note = Description of Artificial Sequence: Synthetic peptide
  VARIANT 1: note = X is any amino acid
  VARIANT 2..3: note = Ile, Val, Leu, B1-Ile, B1-Val, B1-Leu or a dipeptide comprising Gly-Ile or B1-Gly-Ile, wherein B1 represents a first blocking moiety. This region may encompass 1 to 2 residues, wherein some positions may be absent.
  DISULFID 4..14: note = Disulfide bond
  VARIANT 6: note = Independently selected from Trp or analogs of Trp
  VARIANT 9: note = Independently selected from Trp or analogs of Trp
  VARIANT 11: note = His, Ala or an analog of Ala, Phe, Trp or an analog of Trp
  VARIANT 15..17: note = L-Thr, D-Thr, Ile, Val, Gly, a dipeptide selected from Thr-Ala or Thr-Asn, or a tripeptide comprising Thr-Ala-Asn, wherein a C-term -OH of any of the L-Thr, D-Thr, Ile, Val, Gly, Ala or Asn is optionally replaced by a second blocking moiety. This region may encompass 1 to 3 residues, wherein some positions may be absent.
  VARIANT 18: note = X is any amino acid
  REGION 1..18: note = See specification as filed for detailed description of substitutions and preferred embodiments
XXXCVXQDXGXHRCXXXX

SEQ ID NO: 72 - skipped

SEQ ID NO: 73 - protein, 15 aa, synthetic construct
  REGION 1..15: note = Description of Artificial Sequence: Synthetic peptide
  VARIANT 1: note = X is any amino acid
  DISULFID 3..13: note = Disulfide bond
  SITE 5: note = methyl-tryptophan
  SITE 9: note = MeGly
  SITE 14: note = MeIle
  VARIANT 15: note = X is any amino acid
  REGION 1..15: note = See specification as filed for detailed description of substitutions and preferred embodiments
XICVWQDWGAHRCIX

SEQ ID NO: 74 - protein, 15 aa, synthetic construct
  REGION 1..15: note = Description of Artificial Sequence: Synthetic peptide
  VARIANT 1: note = X is any amino acid
  DISULFID 3..13: note = Disulfide bond
  SITE 5: note = Methyl-Tryptophan
  SITE 9: note = MeGly
  SITE 14: note = MeIle
  VARIANT 15: note = X is any amino acid
  REGION 1..15: note = See specification as filed for detailed description of substitutions and preferred embodiments
XICVWQDWGAHRCIX